European Patent Application EP 4 674 863 A1, published January 7, 2026. Title: 一种用于治疗亨廷顿疾病的慢病毒样颗粒. Applicant: 上海本导基因技术有限公司. The sequence listing filed with the application follows.

SEQUENCE LISTING (29 sequences)

SEQ ID NO: 1 - DNA, 10711 bp, synthetic construct
  source 1..10711: mol_type = other DNA
gacggatcgggagatctcccgatcccctatggtgcactctcagtacaatctgctctgatgccgcatagttaagccagtatctgctccctgcttgtgtgttggaggtcgctgagtagtgcgcgagcaaaatttaagctacaacaaggcaaggcttgaccgacaattgcatgaagaatctgcttagggttaggcgttttgcgctgcttcgcgatgtacgggccagatatacgcgttgacattgattattgactagttattaatagtaatcaattacggggtcattagttcatagcccatatatggagttccgcgttacataacttacggtaaatggcccgcctggctgaccgcccaacgacccccgcccattgacgtcaataatgacgtatgttcccatagtaacgccaatagggactttccattgacgtcaatgggtggagtatttacggtaaactgcccacttggcagtacatcaagtgtatcatatgccaagtacgccccctattgacgtcaatgacggtaaatggcccgcctggcattatgcccagtacatgaccttatgggactttcctacttggcagtacatctacgtattagtcatcgctattaccatggtgatgcggttttggcagtacatcaatgggcgtggatagcggtttgactcacggggatttccaagtctccaccccattgacgtcaatgggagtttgttttggcaccaaaatcaacgggactttccaaaatgtcgtaacaactccgccccattgacgcaaatgggcggtaggcgtgtacggtgggaggtctatataagcagagctggtttagtgaaccgtcagatccgctagcgctaccggtcgccaccatggcctctaattttactcaatttgtgcttgtcgataatggggggacgggagatgtgaccgttgcccctagcaatttcgcaaatggcgttgcagaatggatctctagcaacagcagaagccaagcgtacaaagtaacgtgttccgttcgccaaagctccgcccaaaaacggaagtatacaataaaggttgaggtgccgaaagtagccactcaaacagttggtggggtagaattgcccgtagcggcatggcggtcatatctcaatatggaactcactatcccaatcttcgccacgaatagcgattgtgagctgatagttaaggctatgcaaggtcttctcaaagatggaaaccctattccatctgctatcgccgccaacagcgggatatacagccagaactatccgattgtgcagtccggactcagatctcgagctcaagcttcgaattctgcagtcgacggtaccgcgggcccgggatccatggactcgggccgggacttcctgaccctgcacggcctacaggatgatgaggatctacaggcgctgctgaagggcagccagctcctgaaggtgaagtccagctcatggaggagagagcgcttctacaagttgcaggaggactgcaagaccatctggcaggagtcccgcaaggtcatgcggaccccggagtcccagctgttctccatcgaggacattcaggaggtgcgaatggggcaccgcacggagggtctggagaagttcgcccgtgatgtgcccgaggaccgctgcttctccattgtcttcaaggaccagcgcaatacactagacctcatcgccccatcgccagctgatgcccagcactgggtgctggggctgcacaagatcatccaccactcaggctccatggaccagcgtcagaagctacagcactggattcactcctgcttgcgaaaagctgacaaaaacaaggacaacaagatgagcttcaaggagctgcagaacttcctgaaggagctcaacatccagcctcgagccgaattcaccctggccgccagggccagcgtgctgagcggcggcgagctggacaggtgggagaagatcaggctgaggcccggcggcaagaagaagtataagctgaagcacatcgtgtgggccagcagggagctggagaggttcgccgtgaaccccggcctgctggagaccagcgagggctgcaggcagatcctgggccagctgcagcccagcctgcagaccggcagcgaggagctgaggagcctgtacaacaccgtggccaccctgtactgcgtgcaccagaggatcgagatcaaggacaccaaggaggccctggacaagatcgaggaggagcagaacaagtccaagaagaaggcccagcaggccgccgccgacaccggccacagcagccaggtgagccagaactaccccatcgtgcagaacatccagggccagatggtgcaccaggccatcagccccaggaccctgaacgcctgggtgaaggtggtggaggagaaggccttcagccccgaggtgatccccatgttcagcgccctgagcgagggagccaccccccaggacctgaacaccatgctgaacaccgtgggcggccaccaggccgccatgcagatgctgaaggagaccatcaacgaggaggccgccgagtgggacagggtgcaccccgtgcacgccggccccatcgcccccggccagatgagggagccccgcggcagcgacatcgccggcaccaccagcaccctgcaggagcagatcggctggatgaccaacaacccccccatccccgtgggcgaaatctacaagaggtggatcatcctgggcctgaacaagatcgtgaggatgtacagccccaccagcatcctggatatcaggcagggccccaaagagcccttcagggactacgtggacaggttctacaagaccctgcgcgccgagcaggccagccaggaggtgaagaactggatgaccgagaccctgctggtgcagaacgccaaccccgactgcaagaccatcctgaaggccctgggacccgccgccaccctggaggagatgatgaccgcctgccagggcgtgggcggccccggccacaaggccagggtgctggccgaggccatgagccaggtgaccaacaccgccaccatcatgatgcagaggggcaacttcaggaaccagaggaagatggtgaagtgcttcaactgcggcaaggagggccacaccgccaggaactgccgcgcccccaggaagaagggctgctggaagtgcggcaaggagggccaccagatgaaggactgcaccgagaggcaggctaattttttagggaagatctggccttcctacaagggaaggccagggaattttcttcagagcagaccagagccaacagccccaccatttcttcagagcagaccagagccaacagccccaccagaagagagcttcaggtctggggtagagacaacaactccccctcagaagcaggagccgatagacaaggaactgtatcctttaacttccctcagatcactctttggcaacgacccctcgtcacaataaagatcggtggccagctgaaggaggccctgctggacaccggcgccgacgacaccgtgctggaggagatgagcctgcccggcaggtggaagcccaagatgatcggcggcatcggcggcttcatcaaggtgaggcagtacgaccagatcctgatcgagatctgcggccacaaggccatcggcaccgtgctggtgggacctacacctgtgaacatcatcggcaggaacctgctgacccagatcggctgcaccctgaacttccccatcagccccatcgagaccgtgcccgtgaagctgaagcccggcatggacggccctaaggtgaagcagtggcccctgaccgaggagaagatcaaggccctggtggagatctgcaccgagatggagaaggagggcaagatcagcaagatcggccccgagaacccctacaacacccccgtgttcgccatcaagaagaaggacagcaccaagtggaggaagctggtggacttcagggagctgaacaagaggacccaggacttctgggaggtgcagctgggcatcccccaccccgccggcctgaagaagaagaagagcgtgaccgtgctggacgtgggcgacgcctacttcagcgtgcccctggacgaggacttcaggaagtataccgccttcaccatccccagcatcaacaacgagacccccggcatccgctaccagtacaacgtgctgccccagggctggaagggcagccccgccatcttccagagcagcatgacaaagatcctggagcccttcaagaagcagaaccccgacatcgtgatctatcagtacatggacgacctgtacgtgggcagcgacctggagatcggccagcacaggaccaagatcgaggagctgaggcagcacctgctgaggtggggcctgaccacccccgacaagaagcaccagaaggagcccccattcctgtggatgggctacgagctgcaccccgacaagtggaccgtgcagcccatcgtgctgcccgagaaggacagctggaccgtgaacgacattcagaagctggtgggcaagctgaactgggccagccagatctaccctggcatcaaggtgaggcagctgtgcaagctgctgaggggcacaaaggctctgaccgaggtgatccccctgaccgaggaggccgagctggagctggccgagaacagggagatcctgaaggagcccgtgcacggcgtgtactacgaccccagcaaggacctgatcgccgagatccagaagcagggccagggccagtggacctaccagatctaccaggagcccttcaagaacctgaagaccggcaagtacgcccgcatgcgcggcgcccacaccaacgacgtgaagcagctgaccgaggccgtgcagaagatcaccaccgagagcatcgtgatctggggcaagactcctaagttcaagctgcccatccagaaggagacctgggagacctggtggaccgagtactggcaggccacctggattcccgagtgggagttcgtgaacacccctcccctggtgaagctgtggtatcagctggagaaggagcccatcgtgggcgccgagaccttctacgtggacggcgccgccaacagggagaccaagctgggcaaggccggctacgtgaccaacaagggccgccagaaggtggtgcccctgaccaacaccaccaaccagaagaccgagctgcaggctatctacctggccctgcaggactcaggcctggaggtgaacatcgtgaccgacagccagtacgccctgggcatcatccaggcccagcccgacaagagcgagagcgagctggtgaaccagatcatcgagcagctgatcaagaaggagaaggtgtacctggcctgggtgcccgcccacaagggcatcggcggcaacgagcaggtggacaagctggtgagcgccggcatcaggaagatcctgttcctggacggcatcgacaaggcccaggacgagcacgagaagtaccacagcaactggagggctatggctagcgacttcaacctgcctcccgtggtggctaaggagatcgtggccagctgcgacaagtgccagctgaagggcgaggccatgcacggccaggtggactgcagccccggcatctggcagctggtttgcacccacctggagggcaaggtgatcctggtggccgtgcacgtggcctccggctacatcgaggccgaggtgatccccgccgagaccggccaggagaccgcctacttcctgctgaagctggccggccgctggcccgtgaagaccatccacaccgacaacggcagcaacttcaccagcgccaccgtgaaggctgcctgctggtgggccggcatcaagcaggagttcggcatcccctacaacccccagtctcagggcgtggtggagagcatgaacaaggagctgaagaagatcatcggccaggtgagggaccaggccgagcacctgaagaccgccgtgcagatggccgtgttcatccacaacttcaagaggaagggcggcatcggcggctacagcgccggcgagaggatcgtggacatcatcgccaccgacatccagaccaaggagctgcagaagcagatcaccaagatccagaacttcagggtgtactacagggacagcaggaaccctctgtggaagggccccgccaagctgctgtggaagggcgagggcgccgtggtgatccaggacaacagcgacatcaaggtggtgcccaggaggaaggccaagatcatcagggactacggcaagcagatggccggcgacgactgcgtggcctccaggcaggacgaggactgataaggatccctcgagcatgcatctagagggccctattctatagtgtcacctaaatgctagagctcgctgatcagcctcgactgtgccttctagttgccagccatctgttgtttgcccctcccccgtgccttccttgaccctggaaggtgccactcccactgtcctttcctaataaaatgaggaaattgcatcgcattgtctgagtaggtgtcattctattctggggggtggggtggggcaggacagcaagggggaggattgggaagacaatagcaggcatgctggggatgcggtgggctctatggcttctgaggcggaaagaaccagctggggctctagggggtatccccacgcgccctgtagcggcgcattaagcgcggcgggtgtggtggttacgcgcagcgtgaccgctacacttgccagcgccctagcgcccgctcctttcgctttcttcccttcctttctcgccacgttcgccggctttccccgtcaagctctaatcgggggctccctttagggttccgatttagtgctttacggcacctcgaccccaaaaaacttgattagggtgatggttcacgtagtgggccatcgccctgatagacggtttttcgccctttgacgttggagtccacgttctttaatagtggactcttgttccaaactggaacaacactcaaccctatctcggtctattcttttgatttataagggattttgccgatttcggcctattggttaaaaaatgagctgatttaacaaaaatttaacgcgaattaattctgtggaatgtgtgtcagttagggtgtggaaagtccccaggctccccagcaggcagaagtatgcaaagcatgcatctcaattagtcagcaaccaggtgtggaaagtccccaggctccccagcaggcagaagtatgcaaagcatgcatctcaattagtcagcaaccatagtcccgcccctaactccgcccatcccgcccctaactccgcccagttccgcccattctccgccccatggctgactaattttttttatttatgcagaggccgaggccgcctctgcctctgagctattccagaagtagtgaggaggcttttttggaggcctaggcttttgcaaaaagctcccgggagcttgtatatccattttcggatctgatcaagagacaggatgaggatcgtttcgcatgattgaacaagatggattgcacgcaggttctccggccgcttgggtggagaggctattcggctatgactgggcacaacagacaatcggctgctctgatgccgccgtgttccggctgtcagcgcaggggcgcccggttctttttgtcaagaccgacctgtccggtgccctgaatgaactgcaggacgaggcagcgcggctatcgtggctggccacgacgggcgttccttgcgcagctgtgctcgacgttgtcactgaagcgggaagggactggctgctattgggcgaagtgccggggcaggatctcctgtcatctcaccttgctcctgccgagaaagtatccatcatggctgatgcaatgcggcggctgcatacgcttgatccggctacctgcccattcgaccaccaagcgaaacatcgcatcgagcgagcacgtactcggatggaagccggtcttgtcgatcaggatgatctggacgaagagcatcaggggctcgcgccagccgaactgttcgccaggctcaaggcgcgcatgcccgacggcgaggatctcgtcgtgacccatggcgatgcctgcttgccgaatatcatggtggaaaatggccgcttttctggattcatcgactgtggccggctgggtgtggcggaccgctatcaggacatagcgttggctacccgtgatattgctgaagagcttggcggcgaatgggctgaccgcttcctcgtgctttacggtatcgccgctcccgattcgcagcgcatcgccttctatcgccttcttgacgagttcttctgagcgggactctggggttcgaaatgaccgaccaagcgacgcccaacctgccatcacgagatttcgattccaccgccgccttctatgaaaggttgggcttcggaatcgttttccgggacgccggctggatgatcctccagcgcggggatctcatgctggagttcttcgcccaccccaacttgtttattgcagcttataatggttacaaataaagcaatagcatcacaaatttcacaaataaagcatttttttcactgcattctagttgtggtttgtccaaactcatcaatgtatcttatcatgtctgtataccgtcgacctctagctagagcttggcgtaatcatggtcatagctgtttcctgtgtgaaattgttatccgctcacaattccacacaacatacgagccggaagcataaagtgtaaagcctggggtgcctaatgagtgagctaactcacattaattgcgttgcgctcactgcccgctttccagtcgggaaacctgtcgtgccagctgcattaatgaatcggccaacgcgcggggagaggcggtttgcgtattgggcgctcttccgcttcctcgctcactgactcgctgcgctcggtcgttcggctgcggcgagcggtatcagctcactcaaaggcggtaatacggttatccacagaatcaggggataacgcaggaaagaacatgtgagcaaaaggccagcaaaaggccaggaaccgtaaaaaggccgcgttgctggcgtttttccataggctccgcccccctgacgagcatcacaaaaatcgacgctcaagtcagaggtggcgaaacccgacaggactataaagataccaggcgtttccccctggaagctccctcgtgcgctctcctgttccgaccctgccgcttaccggatacctgtccgcctttctcccttcgggaagcgtggcgctttctcatagctcacgctgtaggtatctcagttcggtgtaggtcgttcgctccaagctgggctgtgtgcacgaaccccccgttcagcccgaccgctgcgccttatccggtaactatcgtcttgagtccaacccggtaagacacgacttatcgccactggcagcagccactggtaacaggattagcagagcgaggtatgtaggcggtgctacagagttcttgaagtggtggcctaactacggctacactagaagaacagtatttggtatctgcgctctgctgaagccagttaccttcggaaaaagagttggtagctcttgatccggcaaacaaaccaccgctggtagcggtggtttttttgtttgcaagcagcagattacgcgcagaaaaaaaggatctcaagaagatcctttgatcttttctacggggtctgacgctcagtggaacgaaaactcacgttaagggattttggtcatgagattatcaaaaaggatcttcacctagatccttttaaattaaaaatgaagttttaaatcaatctaaagtatatatgagtaaacttggtctgacagttaccaatgcttaatcagtgaggcacctatctcagcgatctgtctatttcgttcatccatagttgcctgactccccgtcgtgtagataactacgatacgggagggcttaccatctggccccagtgctgcaatgataccgcgagacccacgctcaccggctccagatttatcagcaataaaccagccagccggaagggccgagcgcagaagtggtcctgcaactttatccgcctccatccagtctattaattgttgccgggaagctagagtaagtagttcgccagttaatagtttgcgcaacgttgttgccattgctacaggcatcgtggtgtcacgctcgtcgtttggtatggcttcattcagctccggttcccaacgatcaaggcgagttacatgatcccccatgttgtgcaaaaaagcggttagctccttcggtcctccgatcgttgtcagaagtaagttggccgcagtgttatcactcatggttatggcagcactgcataattctcttactgtcatgccatccgtaagatgcttttctgtgactggtgagtactcaaccaagtcattctgagaatagtgtatgcggcgaccgagttgctcttgcccggcgtcaatacgggataataccgcgccacatagcagaactttaaaagtgctcatcattggaaaacgttcttcggggcgaaaactctcaaggatcttaccgctgttgagatccagttcgatgtaacccactcgtgcacccaactgatcttcagcatcttttactttcaccagcgtttctgggtgagcaaaaacaggaaggcaaaatgccgcaaaaaagggaataagggcgacacggaaatgttgaatactcatactcttcctttttcaatattattgaagcatttatcagggttattgtctcatgagcggatacatatttgaatgtatttagaaaaataaacaaataggggttccgcgcacatttccccgaaaagtgccacctgacgtc

SEQ ID NO: 2 - DNA, 8890 bp, synthetic construct
  source 1..8890: mol_type = other DNA
ggatcccctgagggggcccccatgggctagaggatccggcctcggcctctgcataaataaaaaaaattagtcagccatgagcttggcccattgcatacgttgtatccatatcataatatgtacatttatattggctcatgtccaacattaccgccatgttgacattgattattgactagttattaatagtaatcaattacggggtcattagttcatagcccatatatggagttccgcgttacataacttacggtaaatggcccgcctggctgaccgcccaacgacccccgcccattgacgtcaataatgacgtatgttcccatagtaacgccaatagggactttccattgacgtcaatgggtggagtatttacggtaaactgcccacttggcagtacatcaagtgtatcatatgccaagtacgccccctattgacgtcaatgacggtaaatggcccgcctggcattatgcccagtacatgaccttatgggactttcctacttggcagtacatctacgtattagtcatcgctattaccatggtgatgcggttttggcagtacatcaatgggcgtggatagcggtttgactcacggggatttccaagtctccaccccattgacgtcaatgggagtttgttttggcaccaaaatcaacgggactttccaaaatgtcgtaacaactccgccccattgacgcaaatgggcggtaggcgtgtacggtgggaggtctatataagcagagctcgtttagtgaaccgtcagatcgcctggagacgccatccacgctgttttgacctccatagaagacaccgggaccgatccagcctcccctcgaagcttacatgtggtaccgagctcggatcctgagaacttcagggtgagtctatgggacccttgatgttttctttccccttcttttctatggttaagttcatgtcataggaaggggagaagtaacagggtacacatattgaccaaatcagggtaattttgcatttgtaattttaaaaaatgctttcttcttttaatatacttttttgtttatcttatttctaatactttccctaatctctttctttcagggcaataatgatacaatgtatcatgcctctttgcaccattctaaagaataacagtgataatttctgggttaaggcaatagcaatatttctgcatataaatatttctgcatataaattgtaactgatgtaagaggtttcatattgctaatagcagctacaatccagctaccattctgcttttattttatggttgggataaggctggattattctgagtccaagctaggcccttttgctaatcatgttcatacctcttatcttcctcccacagctcctgggcaacgtgctggtctgtgtgctggcccatcactttggcaaagcacgtgagatctgaattcgagatctgccgccgccatgggtgcgagagcgtcagtattaagcgggggagaattagatcgatgggaaaaaattcggttaaggccagggggaaagaaaaaatataaattaaaacatatagtatgggcaagcagggagctagaacgattcgcagttaatcctggcctgttagaaacatcagaaggctgtagacaaatactgggacagctacaaccatcccttcagacaggatcagaagaacttagatcattatataatacagtagcaaccctctattgtgtgcatcaaaggatagagataaaagacaccaaggaagctttagacaagatagaggaagagcaaaacaaaagtaagaaaaaagcacagcaagcagcagctgacacaggacacagcaatcaggtcagccaaaattaccctatagtgcagaacatccaggggcaaatggtacatcaggccatatcacctagaactttaaatgcatgggtaaaagtagtagaagagaaggctttcagcccagaagtgatacccatgttttcagcattatcagaaggagccaccccacaagatttaaacaccatgctaaacacagtggggggacatcaagcagccatgcaaatgttaaaagagaccatcaatgaggaagctgcagaatgggatagagtgcatccagtgcatgcagggcctattgcaccaggccagatgagagaaccaaggggaagtgacatagcaggaactactagtacccttcaggaacaaataggatggatgacacataatccacctatcccagtaggagaaatctataaaagatggataatcctgggattaaataaaatagtaagaatgtatagccctaccagcattctggacataagacaaggaccaaaggaaccctttagagactatgtagaccgattctataaaactctaagagccgagcaagcttcacaagaggtaaaaaattggatgacagaaaccttgttggtccaaaatgcgaacccagattgtaagactattttaaaagcattgggaccaggagcgacactagaagaaatgatgacagcatgtcagggagtggggggacccggccataaagcaagagttttggctgaagcaatgagccaagtaacaaatccagctaccataatgatacagaaaggcaattttaggaaccaaagaaagactgttaagtgtttcaattgtggcaaagaagggcacatagccaaaaattgcagggcccctaggaaaaagggctgttggaaatgtggaaaggaaggacaccaaatgaaagattgtactgagagacaggctaattttttagggaagatctggccttcccacaagggaaggccagggaattttcttcagagcagaccagagccaacagccccaccagaagagagcttcaggtttggggaagagacaacaactccctctcagaagcaggagccgatagacaaggaactgtatcctttagcttccctcagatcactctttggcagcgacccctcgtcacaataaagataggggggcaattaaaggaagctctattagatacaggagcagatgatacagtattagaagaaatgaatttgccaggaagatggaaaccaaaaatgatagggggaattggaggttttatcaaagtaagacagtatgatcagatactcatagaaatctgtggacataaagctataggtacagtattagtaggacctacacctgtcaacataattggaagaaatctgttgactcagattggttgcactttaaattttcccattagccctattgagactgtaccagtaaaattaaagccaggaatggatggcccaaaagttaaacaatggccattgacagaagaaaaaataaaagcattagtagaaatttgtacagagatggaaaaggaagggaaaatttcaaaaattgggcctgaaaatccatacaatactccagtatttgccataaagaaaaaagacagtactaaatggagaaaattagtagatttcagagaacttaataagagaactcaagacttctgggaagttcaattaggaataccacatcccgcagggttaaaaaagaaaaaatcagtaacagtactggatgtgggtgatgcatatttttcagttcccttagatgaagacttcaggaaatatactgcatttaccatacctagtataaacaatgagacaccagggattagatatcagtacaatgtgcttccacagggatggaaaggatcaccagcaatattccaaagtagcatgacaaaaatcttagagccttttagaaaacaaaatccagacatagttatctatcaatacatggatgatttgtatgtaggatctgacttagaaatagggcagcatagaacaaaaatagaggagctgagacaacatctgttgaggtggggacttaccacaccagacaaaaaacatcagaaagaacctccattcctttggatgggttatgaactccatcctgataaatggacagtacagcctatagtgctgccagaaaaagacagctggactgtcaatgacatacagaagttagtggggaaattgaattgggcaagtcagatttacccagggattaaagtaaggcaattatgtaaactccttagaggaaccaaagcactaacagaagtaataccactaacagaagaagcagagctagaactggcagaaaacagagagattctaaaagaaccagtacatggagtgtattatgacccatcaaaagacttaatagcagaaatacagaagcaggggcaaggccaatggacatatcaaatttatcaagagccatttaaaaatctgaaaacaggaaaatatgcaagaatgaggggtgcccacactaatgatgtaaaacaattaacagaggcagtgcaaaaaataaccacagaaagcatagtaatatggggaaagactcctaaatttaaactgcccatacaaaaggaaacatgggaaacatggtggacagagtattggcaagccacctggattcctgagtgggagtttgttaatacccctcctttagtgaaattatggtaccagttagagaaagaacccatagtaggagcagaaaccttctatgtagatggggcagctaacagggagactaaattaggaaaagcaggatatgttactaatagaggaagacaaaaagttgtcaccctaactgacacaacaaatcagaagactgagttacaagcaatttatctagctttgcaggattcgggattagaagtaaacatagtaacagactcacaatatgcattaggaatcattcaagcacaaccagatcaaagtgaatcagagttagtcaatcaaataatagagcagttaataaaaaaggaaaaggtctatctggcatgggtaccagcacacaaaggaattggaggaaatgaacaagtagataaattagtcagtgctggaatcaggaaagtactatttttagatggaatcgataaggctcaagaagaacacgaaaagtaccactctaattggagagccatggcaagtgattttaacctgccacctgtagtagcaaaagaaatagtagccagctgtgataaatgtcagctaaaaggagaagccatgcatggacaagtagactgtagtccaggaatatggcaactagtttgtacacatctagaaggaaaaattatcctggtagcagttcatgtagccagtggatatatagaagcagaagttattccagcagagacagggcaggaaacagcatattttctcttaaaattagcaggaagatggccagtaaaaacaatacatacagacaatggcagcaatttcaccagtactacggttaaggccgcctgttggtgggcagggatcaagcaggaatttggcattccctacaatccccaaagccaaggagtagtagaatctatgaataatgaattaaagaaaattataggacaggtaagagatcaggctgaacaccttaagacagcagtacaaatggcagtattcatccacaattttaaaagaaaaggggggattggggggtacagtgcaggggaaagaatagtagacataatagcaacagacatacaaactaaagaattacaaaaacaaattacaaaaattcaaaattttcgggtttattacagggacagcagagatccagtttggaaaggaccagcaaagctcctctggaaaggtgaaggggcagtagtaatacaagataatagtgacataaaagtagtgccaagaagaaaagcaaagatcatcagggattatggaaaacagatggcaggtgatgattgtgtggcaagtagacaggatgaggattaacacatggaattccggagcggccgcaggagctttgttccttgggttcttgggagcagcaggaagcactatgggcgcagcgtcaatgacgctgacggtacaggccagacaattattgtctggtatagtgcagcagcagaacaatttgctgagggctattgaggcgcaacagcatctgttgcaactcacagtctggggcatcaagcagctccaggcaagaatcctggctgtggaaagatacctaaaggatcaacagctcctggggatttggggttgctctggaaaactcatttgcaccactgctgtgccttggaatgctagttggagtaataaatctctggaacagatttggaatcacacgacctggatggagtgggacagagaaattaacaattacacaagcttccgcggaattcaccccaccagtgcaggctgcctatcagaaagtggtggctggtgtggctaatgccctggcccacaagtatcactaagctcgctttcttgctgtccaatttctattaaaggttcctttgttccctaagtccaactactaaactgggggatattatgaagggccttgagcatctggattctgcctaataaaaaacatttattttcattgcaatgatgtatttaaattatttctgaatattttactaaaaagggaatgtgggaggtcagtgcatttaaaacataaagaaatgaagagctagttcaaaccttgggaaaatacactatatcttaaactccatgaaagaaggtgaggctgcaaacagctaatgcacattggcaacagcccctgatgcctatgccttattcatccctcagaaaaggattcaagtagaggcttgatttggaggttaaagttttgctatgctgtattttacattacttattgttttagctgtcctcatgaatgtcttttcactacccatttgcttatcctgcatctctcagccttgactccactcagttctcttgcttagagataccacctttcccctgaagtgttccttccatgttttacggcgagatggtttctcctcgcctggccactcagccttagttgtctctgttgtcttatagaggtctacttgaagaaggaaaaacagggggcatggtttgactgtcctgtgagcccttcttccctgcctcccccactcacagtgacccggaatccctcgacatggcagtctagcactagtgcggccgcagatctgcttcctcgctcactgactcgctgcgctcggtcgttcggctgcggcgagcggtatcagctcactcaaaggcggtaatacggttatccacagaatcaggggataacgcaggaaagaacatgtgagcaaaaggccagcaaaaggccaggaaccgtaaaaaggccgcgttgctggcgtttttccataggctccgcccccctgacgagcatcacaaaaatcgacgctcaagtcagaggtggcgaaacccgacaggactataaagataccaggcgtttccccctggaagctccctcgtgcgctctcctgttccgaccctgccgcttaccggatacctgtccgcctttctcccttcgggaagcgtggcgctttctcatagctcacgctgtaggtatctcagttcggtgtaggtcgttcgctccaagctgggctgtgtgcacgaaccccccgttcagcccgaccgctgcgccttatccggtaactatcgtcttgagtccaacccggtaagacacgacttatcgccactggcagcagccactggtaacaggattagcagagcgaggtatgtaggcggtgctacagagttcttgaagtggtggcctaactacggctacactagaagaacagtatttggtatctgcgctctgctgaagccagttaccttcggaaaaagagttggtagctcttgatccggcaaacaaaccaccgctggtagcggtggtttttttgtttgcaagcagcagattacgcgcagaaaaaaaggatctcaagaagatcctttgatcttttctacggggtctgacgctcagtggaacgaaaactcacgttaagggattttggtcatgagattatcaaaaaggatcttcacctagatccttttaaattaaaaatgaagttttaaatcaatctaaagtatatatgagtaaacttggtctgacagttaccaatgcttaatcagtgaggcacctatctcagcgatctgtctatttcgttcatccatagttgcctgactccccgtcgtgtagataactacgatacgggagggcttaccatctggccccagtgctgcaatgataccgcgagacccacgctcaccggctccagatttatcagcaataaaccagccagccggaagggccgagcgcagaagtggtcctgcaactttatccgcctccatccagtctattaattgttgccgggaagctagagtaagtagttcgccagttaatagtttgcgcaacgttgttgccattgctacaggcatcgtggtgtcacgctcgtcgtttggtatggcttcattcagctccggttcccaacgatcaaggcgagttacatgatcccccatgttgtgcaaaaaagcggttagctccttcggtcctccgatcgttgtcagaagtaagttggccgcagtgttatcactcatggttatggcagcactgcataattctcttactgtcatgccatccgtaagatgcttttctgtgactggtgagtactcaaccaagtcattctgagaatagtgtatgcggcgaccgagttgctcttgcccggcgtcaatacgggataataccgcgccacatagcagaactttaaaagtgctcatcattggaaaacgttcttcggggcgaaaactctcaaggatcttaccgctgttgagatccagttcgatgtaacccactcgtgcacccaactgatcttcagcatcttttactttcaccagcgtttctgggtgagcaaaaacaggaaggcaaaatgccgcaaaaaagggaataagggcgacacggaaatgttgaatactcatactcttcctttttcaatattattgaagcatttatcagggttattgtctcatgagcggatacatatttgaatgtatttagaaaaataaacaaataggggttccgcgcacatttccccgaaaagtgccacctgacgt

SEQ ID NO: 3 - DNA, 7910 bp, synthetic construct
  source 1..7910: mol_type = other DNA
tcgcgcgtttcggtgatgacggtgaaaacctctgacacatgcagctcccggagacggtcacagcttgtctgtaagcggatgccgggagcagacaagcccgtcagggcgcgtcagcgggtgttggcgggtgtcggggctggcttaactatgcggcatcagagcagattgtactgagagtgcaccatatgcggtgtgaaataccgcacagatgcgtaaggagaaaataccgcatcaggcgccattcgccattcaggctgcgcaactgttgggaagggcgatcggtgcgggcctcttcgctattacgccagctggcgaaagggggatgtgctgcaaggcgattaagttgggtaacgccagggttttcccagtcacgacgttgtaaaacgacggccagtgaattcgagcttgcatgcctgcaggtcgttacataacttacggtaaatggcccgcctggctgaccgcccaacgacccccgcccattgacgtcaataatgacgtatgttcccatagtaacgccaatagggactttccattgacgtcaatgggtggactatttacggtaaactgcccacttggcagtacatcaagtgtatcatatgccaagtacgccccctattgacgtcaatgacggtaaatggcccgcctggcattatgcccagtacatgaccttatgggactttcctacttggcagtacatctacgtattagtcatcgctattaccatggtgatgcggttttggcagtacatcaatgggcgtggatagcggtttgactcacggggatttccaagtctccaccccattgacgtcaatgggagtttgttttggcaccaaaatcaacgggactttccaaaatgtcgtaacaactccgccccattgacgcaaatgggcggtaggcgtgtacggtgggaggtctatataagcagagctcgtttagtgaaccgtcagatcgcctggagacgccatccacgctgttttgacctccatagaagacaccgggaccgatccagcctccggactctagaggatccggtactcgaggaactgaaaaaccagaaagttaactggtaagtttagtctttttgtcttttatttcaggtcccgatccggtggtggtgcaaatcaaagaactgctcctcagtggatgttgcctttacttctaggcctgtacggaagtgttacttctgctctaaaagctgcggaattgtacccgcggacgcgtgccaccatggccccaaagaagaagcggaaggtcggtatccacggagtcccagcagccgacaagaagtacagcatcggcctggacatcggcaccaactctgtgggctgggccgtgatcaccgacgagtacaaggtgcccagcaagaaattcaaggtgctgggcaacaccgaccggcacagcatcaagaagaacctgatcggagccctgctgttcgacagcggcgaaacagccgaggccacccggctgaagagaaccgccagaagaagatacaccagacggaagaaccggatctgctatctgcaagagatcttcagcaacgagatggccaaggtggacgacagcttcttccacagactggaagagtccttcctggtggaagaggataagaagcacgagcggcaccccatcttcggcaacatcgtggacgaggtggcctaccacgagaagtaccccaccatctaccacctgagaaagaaactggtggacagcaccgacaaggccgacctgcggctgatctatctggccctggcccacatgatcaagttccggggccacttcctgatcgagggcgacctgaaccccgacaacagcgacgtggacaagctgttcatccagctggtgcagacctacaaccagctgttcgaggaaaaccccatcaacgccagcggcgtggacgccaaggccatcctgtctgccagactgagcaagagcagacggctggaaaatctgatcgcccagctgcccggcgagaagaagaatggcctgttcggaaacctgattgccctgagcctgggcctgacccccaacttcaagagcaacttcgacctggccgaggatgccaaactgcagctgagcaaggacacctacgacgacgacctggacaacctgctggcccagatcggcgaccagtacgccgacctgtttctggccgccaagaacctgtccgacgccatcctgctgagcgacatcctgagagtgaacaccgagatcaccaaggcccccctgagcgcctctatgatcaagagatacgacgagcaccaccaggacctgaccctgctgaaagctctcgtgcggcagcagctgcctgagaagtacaaagagattttcttcgaccagagcaagaacggctacgccggctacattgacggcggagccagccaggaagagttctacaagttcatcaagcccatcctggaaaagatggacggcaccgaggaactgctcgtgaagctgaacagagaggacctgctgcggaagcagcggaccttcgacaacggcagcatcccccaccagatccacctgggagagctgcacgccattctgcggcggcaggaagatttttacccattcctgaaggacaaccgggaaaagatcgagaagatcctgaccttccgcatcccctactacgtgggccctctggccaggggaaacagcagattcgcctggatgaccagaaagagcgaggaaaccatcaccccctggaacttcgaggaagtggtggacaagggcgcttccgcccagagcttcatcgagcggatgaccaacttcgataagaacctgcccaacgagaaggtgctgcccaagcacagcctgctgtacgagtacttcaccgtgtataacgagctgaccaaagtgaaatacgtgaccgagggaatgagaaagcccgccttcctgagcggcgagcagaaaaaggccatcgtggacctgctgttcaagaccaaccggaaagtgaccgtgaagcagctgaaagaggactacttcaagaaaatcgagtgcttcgactccgtggaaatctccggcgtggaagatcggttcaacgcctccctgggcacataccacgatctgctgaaaattatcaaggacaaggacttcctggacaatgaggaaaacgaggacattctggaagatatcgtgctgaccctgacactgtttgaggacagagagatgatcgaggaacggctgaaaacctatgcccacctgttcgacgacaaagtgatgaagcagctgaagcggcggagatacaccggctggggcaggctgagccggaagctgatcaacggcatccgggacaagcagtccggcaagacaatcctggatttcctgaagtccgacggcttcgccaacagaaacttcatgcagctgatccacgacgacagcctgacctttaaagaggacatccagaaagcccaggtgtccggccagggcgatagcctgcacgagcacattgccaatctggccggcagccccgccattaagaagggcatcctgcagacagtgaaggtggtggacgagctcgtgaaagtgatgggccggcacaagcccgagaacatcgtgatcgaaatggccagagagaaccagaccacccagaagggacagaagaacagccgcgagagaatgaagcggatcgaagagggcatcaaagagctgggcagccagatcctgaaagaacaccccgtggaaaacacccagctgcagaacgagaagctgtacctgtactacctgcagaatgggcgggatatgtacgtggaccaggaactggacatcaaccggctgtccgactacgatgtggaccatatcgtgcctcagagctttctgaaggacgactccatcgacaacaaggtgctgaccagaagcgacaagaaccggggcaagagcgacaacgtgccctccgaagaggtcgtgaagaagatgaagaactactggcggcagctgctgaacgccaagctgattacccagagaaagttcgacaatctgaccaaggccgagagaggcggcctgagcgaactggataaggccggcttcatcaagagacagctggtggaaacccggcagatcacaaagcacgtggcacagatcctggactcccggatgaacactaagtacgacgagaatgacaagctgatccgggaagtgaaagtgatcaccctgaagtccaagctggtgtccgatttccggaaggatttccagttttacaaagtgcgcgagatcaacaactaccaccacgcccacgacgcctacctgaacgccgtcgtgggaaccgccctgatcaaaaagtaccctaagctggaaagcgagttcgtgtacggcgactacaaggtgtacgacgtgcggaagatgatcgccaagagcgagcaggaaatcggcaaggctaccgccaagtacttcttctacagcaacatcatgaactttttcaagaccgagattaccctggccaacggcgagatccggaagcggcctctgatcgagacaaacggcgaaaccggggagatcgtgtgggataagggccgggattttgccaccgtgcggaaagtgctgagcatgccccaagtgaatatcgtgaaaaagaccgaggtgcagacaggcggcttcagcaaagagtctatcctgcccaagaggaacagcgataagctgatcgccagaaagaaggactgggaccctaagaagtacggcggcttcgacagccccaccgtggcctattctgtgctggtggtggccaaagtggaaaagggcaagtccaagaaactgaagagtgtgaaagagctgctggggatcaccatcatggaaagaagcagcttcgagaagaatcccatcgactttctggaagccaagggctacaaagaagtgaaaaaggacctgatcatcaagctgcctaagtactccctgttcgagctggaaaacggccggaagagaatgctggcctctgccggcgaactgcagaagggaaacgaactggccctgccctccaaatatgtgaacttcctgtacctggccagccactatgagaagctgaagggctcccccgaggataatgagcagaaacagctgtttgtggaacagcacaagcactacctggacgagatcatcgagcagatcagcgagttctccaagagagtgatcctggccgacgctaatctggacaaagtgctgtccgcctacaacaagcaccgggataagcccatcagagagcaggccgagaatatcatccacctgtttaccctgaccaatctgggagcccctgccgccttcaagtactttgacaccaccatcgaccggaagaggtacaccagcaccaaagaggtgctggacgccaccctgatccaccagagcatcaccggcctgtacgagacacggatcgacctgtctcagctgggaggcgacaaaaggccggcggccacgaaaaaggccggccaggcaaaaaagaaaaagtaaaattggccgcggggatccagacatgataagatacattgatgagtttggacaaaccacaactagaatgcagtgaaaaaaatgctttatttgtgaaatttgtgatgctattgctttatttgtaaccattataagctgcaataaacaagttaacaacaacaattgcattcattttatgtttcaggttcagggggaggtgtgggaggttttttcggatcctctagagtcgacctgcaggcatgcaagcttggcgtaatcatggtcatagctgtttcctgtgtgaaattgttatccgctcacaattccacacaacatacgagccggaagcataaagtgtaaagcctggggtgcctaatgagtgagctaactcacattaattgcgttgcgctcactgcccgctttccagtcgggaaacctgtcgtgccagctgcattaatgaatcggccaacgcgcggggagaggcggtttgcgtattgggcgctcttccgcttcctcgctcactgactcgctgcgctcggtcgttcggctgcggcgagcggtatcagctcactcaaaggcggtaatacggttatccacagaatcaggggataacgcaggaaagaacatgtgagcaaaaggccagcaaaaggccaggaaccgtaaaaaggccgcgttgctggcgtttttccataggctccgcccccctgacgagcatcacaaaaatcgacgctcaagtcagaggtggcgaaacccgacaggactataaagataccaggcgtttccccctggaagctccctcgtgcgctctcctgttccgaccctgccgcttaccggatacctgtccgcctttctcccttcgggaagcgtggcgctttctcatagctcacgctgtaggtatctcagttcggtgtaggtcgttcgctccaagctgggctgtgtgcacgaaccccccgttcagcccgaccgctgcgccttatccggtaactatcgtcttgagtccaacccggtaagacacgacttatcgccactggcagcagccactggtaacaggattagcagagcgaggtatgtaggcggtgctacagagttcttgaagtggtggcctaactacggctacactagaaggacagtatttggtatctgcgctctgctgaagccagttaccttcggaaaaagagttggtagctcttgatccggcaaacaaaccaccgctggtagcggtggtttttttgtttgcaagcagcagattacgcgcagaaaaaaaggatctcaagaagatcctttgatcttttctacggggtctgacgctcagtggaacgaaaactcacgttaagggattttggtcatgagattatcaaaaaggatcttcacctagatccttttaaattaaaaatgaagttttaaatcaatctaaagtatatatgagtaaacttggtctgacagttaccaatgcttaatcagtgaggcacctatctcagcgatctgtctatttcgttcatccatagttgcctgactccccgtcgtgtagataactacgatacgggagggcttaccatctggccccagtgctgcaatgataccgcgagacccacgctcaccggctccagatttatcagcaataaaccagccagccggaagggccgagcgcagaagtggtcctgcaactttatccgcctccatccagtctattaattgttgccgggaagctagagtaagtagttcgccagttaatagtttgcgcaacgttgttgccattgctacaggcatcgtggtgtcacgctcgtcgtttggtatggcttcattcagctccggttcccaacgatcaaggcgagttacatgatcccccatgttgtgcaaaaaagcggttagctccttcggtcctccgatcgttgtcagaagtaagttggccgcagtgttatcactcatggttatggcagcactgcataattctcttactgtcatgccatccgtaagatgcttttctgtgactggtgagtactcaaccaagtcattctgagaatagtgtatgcggcgaccgagttgctcttgcccggcgtcaatacgggataataccgcgccacatagcagaactttaaaagtgctcatcattggaaaacgttcttcggggcgaaaactctcaaggatcttaccgctgttgagatccagttcgatgtaacccactcgtgcacccaactgatcttcagcatcttttactttcaccagcgtttctgggtgagcaaaaacaggaaggcaaaatgccgcaaaaaagggaataagggcgacacggaaatgttgaatactcatactcttcctttttcaatattattgaagcatttatcagggttattgtctcatgagcggatacatatttgaatgtatttagaaaaataaacaaataggggttccgcgcacatttccccgaaaagtgccacctgacgtctaagaaaccattattatcatgacattaacctataaaaataggcgtatcacgaggccctttcgtc

SEQ ID NO: 4 - DNA, 3172 bp, synthetic construct
  source 1..3172: mol_type = other DNA
tcgcgcgtttcggtgatgacggtgaaaacctctgacacatgcagctcccggagaccgtcacagcttgtctgtaagcggatgccgggagcagacaagcccgtcagggcgcgtcagcgggtgttggcgggtgtcggggctggcttaactatgcggcatcagagcagattgtactgagagtgcaccatatgcggtgtgaaataccgcacagatgcgtaaggagaaaataccgcatcaggcgccattcgccattcaggctgcgcaactgttgggaagggcgatcggtgcgggcctcttcgctattacgccagctggcgaaagggggatgtgctgcaaggcgattaagttgggtaacgccagggttttcccagtcacgacgttgtaaaacgacggccagtgaattcgagggcctatttcccatgattccttcatatttgcatatacgatacaaggctgttagagagataattggaattaatttgactgtaaacacaaagatattagtacaaaatacgtgacgtagaaagtaataatttcttgggtagtttgcagttttaaaattatgttttaaaatggactatcatatgcttaccgtaacttgaaagtatttcgatttcttggctttatatatcttgtggaaaggacgaaacaccggagacgggataccgtctctgtttcagagctaggccaacatgaggatcacccatgtctgcagggcctgctggaaacagcatagcaagttgaaataaggctagtccgttatcaacttggccaacatgaggatcacccatgtctgcagggccgaaaaagtggcaccgagtcggtgctttttttccgcggggatccagacacaattgcattcattttatgtttcaggttcagggggaggtgtgggaggttttttcggatcctctagagtcgacctgcaggcatgcaagcttggcgtaatcatggtcatagctgtttcctgtgtgaaattgttatccgctcacaattccacacaacatacgagccggaagcataaagtgtaaagcctggggtgcctaatgagtgagctaactcacattaattgcgttgcgctcactgcccgctttccagtcgggaaacctgtcgtgccagctgcattaatgaatcggccaacgcgcggggagaggcggtttgcgtattgggcgctcttccgcttcctcgctcactgactcgctgcgctcggtcgttcggctgcggcgagcggtatcagctcactcaaaggcggtaatacggttatccacagaatcaggggataacgcaggaaagaacatgtgagcaaaaggccagcaaaaggccaggaaccgtaaaaaggccgcgttgctggcgtttttccataggctccgcccccctgacgagcatcacaaaaatcgacgctcaagtcagaggtggcgaaacccgacaggactataaagataccaggcgtttccccctggaagctccctcgtgcgctctcctgttccgaccctgccgcttaccggatacctgtccgcctttctcccttcgggaagcgtggcgctttctcatagctcacgctgtaggtatctcagttcggtgtaggtcgttcgctccaagctgggctgtgtgcacgaaccccccgttcagcccgaccgctgcgccttatccggtaactatcgtcttgagtccaacccggtaagacacgacttatcgccactggcagcagccactggtaacaggattagcagagcgaggtatgtaggcggtgctacagagttcttgaagtggtggcctaactacggctacactagaaggacagtatttggtatctgcgctctgctgaagccagttaccttcggaaaaagagttggtagctcttgatccggcaaacaaaccaccgctggtagcggtggtttttttgtttgcaagcagcagattacgcgcagaaaaaaaggatctcaagaagatcctttgatcttttctacggggtctgacgctcagtggaacgaaaactcacgttaagggattttggtcatgagattatcaaaaaggatcttcacctagatccttttaaattaaaaatgaagttttaaatcaatctaaagtatatatgagtaaacttggtctgacagttaccaatgcttaatcagtgaggcacctatctcagcgatctgtctatttcgttcatccatagttgcctgactccccgtcgtgtagataactacgatacgggagggcttaccatctggccccagtgctgcaatgataccgcgagacccacgctcaccggctccagatttatcagcaataaaccagccagccggaagggccgagcgcagaagtggtcctgcaactttatccgcctccatccagtctattaattgttgccgggaagctagagtaagtagttcgccagttaatagtttgcgcaacgttgttgccattgctacaggcatcgtggtgtcacgctcgtcgtttggtatggcttcattcagctccggttcccaacgatcaaggcgagttacatgatcccccatgttgtgcaaaaaagcggttagctccttcggtcctccgatcgttgtcagaagtaagttggccgcagtgttatcactcatggttatggcagcactgcataattctcttactgtcatgccatccgtaagatgcttttctgtgactggtgagtactcaaccaagtcattctgagaatagtgtatgcggcgaccgagttgctcttgcccggcgtcaatacgggataataccgcgccacatagcagaactttaaaagtgctcatcattggaaaacgttcttcggggcgaaaactctcaaggatcttaccgctgttgagatccagttcgatgtaacccactcgtgcacccaactgatcttcagcatcttttactttcaccagcgtttctgggtgagcaaaaacaggaaggcaaaatgccgcaaaaaagggaataagggcgacacggaaatgttgaatactcatactcttcctttttcaatattattgaagcatttatcagggttattgtctcatgagcggatacatatttgaatgtatttagaaaaataaacaaataggggttccgcgcacatttccccgaaaagtgccacctgacgtctaagaaaccattattatcatgacattaacctataaaaataggcgtatcacgaggccctttagtc

SEQ ID NO: 5 - DNA, 5813 bp, synthetic construct
  source 1..5813: mol_type = other DNA
ggatcccctgagggggcccccatgggctagaggatccggcctcggcctctgcataaataaaaaaaattagtcagccatgagcttggcccattgcatacgttgtatccatatcataatatgtacatttatattggctcatgtccaacattaccgccatgttgacattgattattgactagttattaatagtaatcaattacggggtcattagttcatagcccatatatggagttccgcgttacataacttacggtaaatggcccgcctggctgaccgcccaacgacccccgcccattgacgtcaataatgacgtatgttcccatagtaacgccaatagggactttccattgacgtcaatgggtggagtatttacggtaaactgcccacttggcagtacatcaagtgtatcatatgccaagtacgccccctattgacgtcaatgacggtaaatggcccgcctggcattatgcccagtacatgaccttatgggactttcctacttggcagtacatctacgtattagtcatcgctattaccatggtgatgcggttttggcagtacatcaatgggcgtggatagcggtttgactcacggggatttccaagtctccaccccattgacgtcaatgggagtttgttttggcaccaaaatcaacgggactttccaaaatgtcgtaacaactccgccccattgacgcaaatgggcggtaggcgtgtacggtgggaggtctatataagcagagctcgtttagtgaaccgtcagatcgcctggagacgccatccacgctgttttgacctccatagaagacaccgggaccgatccagcctcccctcgaagcttacatgtggtaccgagctcggatcctgagaacttcagggtgagtctatgggacccttgatgttttctttccccttcttttctatggttaagttcatgtcataggaaggggagaagtaacagggtacacatattgaccaaatcagggtaattttgcatttgtaattttaaaaaatgctttcttcttttaatatacttttttgtttatcttatttctaatactttccctaatctctttctttcagggcaataatgatacaatgtatcatgcctctttgcaccattctaaagaataacagtgataatttctgggttaaggcaatagcaatatttctgcatataaatatttctgcatataaattgtaactgatgtaagaggtttcatattgctaatagcagctacaatccagctaccattctgcttttattttatggttgggataaggctggattattctgagtccaagctaggcccttttgctaatcatgttcatacctcttatcttcctcccacagctcctgggcaacgtgctggtctgtgtgctggcccatcactttggcaaagcacgtgagatctgaattctgacactatggactggacctggatcctgttcctggtggccgccgccacccgcgtgcacagcaagttccctatctacacaattccagataaactgggaccctggagccccattgatattcatcatctgagctgccccaataacctggtggtggaggacgagggctgcaccaatctgagcggcttttcctacatggaactgaaggtgggctacatcagcgccatcaagatgaacggcttcacctgcaccggcgtggtgaccgaggccgagacctacaccaatttcgtgggctacgtgaccaccaccttcaagaggaagcacttccggcccacccccgacgcctgcagagccgcctacaactggaagatggccggcgacccacggtacgaggagagcctgcacaacccttaccccgactatcactggctgaggaccgtgaaaaccaccaaggagagcctcgtgatcatcagccccagcgtggccgacctggacccctacgacagatccctgcacagccccgtgtttcccggcggcaactgtagcggcgtggccgtgagctccacctactgcagcaccaaccacgactacaccatctggatgcccgaaaaccctaggctgggcatgagctgcgacatcttcaccaattccagaggcaagcgggcctccaaggggtccgagacctgtggcttcgtggacgagagaggcctgtacaagagcctgaaaggcgcctgcaagctgaagctgtgcggcgtgctgggcctgaggctgatggacggcacctgggtggcaatgcagaccagcaacgagaccaagtggtgcccccccggccagttggtgaatctgcacgactttaggtctgatgagattgaacacctggtggttgaggaactggtgaaaaagagggaggaatgcctggatgccctggagtccatcatgacaactaaaagcgtgtcttttaggagactgagccacctgagaaagctggtgcctggatttggaaaggcctacactatttttaataagaccctgatggaggctgatgctcactacaagtctgtgagaacttggaatgaaatcatcccttctaaaggctgtctgagagtgggcggcagatgtcacccacacgtgaatggcgtgttctttaacggcattatcctgggcccagatggcaatgtgctgatccctgagatgcagagctccctgctgcagcaacacatggaactgctggtgagcagcgtgatccctctgatgcaccccctggccgatcccagcaccgtgtttaagaatggcgatgaggccgaggattttgtggaggtgcaccttcccgatgtgcacgaacggatctcaggagttgacttgggtctcccgaactgggggaagtatgtattactgagtgcaggggccctgactgccttgatgttgataattttcctgatgacatgctggcgagttggtatccatctttgcattaaattaaagcacaccaagaaaagacagatttatacagacatagagatgaaccgacttggaaagtaactcaaatcctgcacaacagattcttcatgtttggaccaaatcaacttgtgataccatgctcaaagaggcctcaattatatttgagtttttaatttttatgaaaaaaaaaaaaaaaaacggaattcaccccaccagtgcaggctgcctatcagaaagtggtggctggtgtggctaatgccctggcccacaagtatcactaagctcgctttcttgctgtccaatttctattaaaggttcctttgttccctaagtccaactactaaactgggggatattatgaagggccttgagcatctggattctgcctaataaaaaacatttattttcattgcaatgatgtatttaaattatttctgaatattttactaaaaagggaatgtgggaggtcagtgcatttaaaacataaagaaatgaagagctagttcaaaccttgggaaaatacactatatcttaaactccatgaaagaaggtgaggctgcaaacagctaatgcacattggcaacagcccctgatgcctatgccttattcatccctcagaaaaggattcaagtagaggcttgatttggaggttaaagttttgctatgctgtattttacattacttattgttttagctgtcctcatgaatgtcttttcactacccatttgcttatcctgcatctctcagccttgactccactcagttctcttgcttagagataccacctttcccctgaagtgttccttccatgttttacggcgagatggtttctcctcgcctggccactcagccttagttgtctctgttgtcttatagaggtctacttgaagaaggaaaaacagggggcatggtttgactgtcctgtgagcccttcttccctgcctcccccactcacagtgacccggaatccctcgacatggcagtctagcactagtgcggccgcagatctgcttcctcgctcactgactcgctgcgctcggtcgttcggctgcggcgagcggtatcagctcactcaaaggcggtaatacggttatccacagaatcaggggataacgcaggaaagaacatgtgagcaaaaggccagcaaaaggccaggaaccgtaaaaaggccgcgttgctggcgtttttccataggctccgcccccctgacgagcatcacaaaaatcgacgctcaagtcagaggtggcgaaacccgacaggactataaagataccaggcgtttccccctggaagctccctcgtgcgctctcctgttccgaccctgccgcttaccggatacctgtccgcctttctcccttcgggaagcgtggcgctttctcatagctcacgctgtaggtatctcagttcggtgtaggtcgttcgctccaagctgggctgtgtgcacgaaccccccgttcagcccgaccgctgcgccttatccggtaactatcgtcttgagtccaacccggtaagacacgacttatcgccactggcagcagccactggtaacaggattagcagagcgaggtatgtaggcggtgctacagagttcttgaagtggtggcctaactacggctacactagaagaacagtatttggtatctgcgctctgctgaagccagttaccttcggaaaaagagttggtagctcttgatccggcaaacaaaccaccgctggtagcggtggtttttttgtttgcaagcagcagattacgcgcagaaaaaaaggatctcaagaagatcctttgatcttttctacggggtctgacgctcagtggaacgaaaactcacgttaagggattttggtcatgagattatcaaaaaggatcttcacctagatccttttaaattaaaaatgaagttttaaatcaatctaaagtatatatgagtaaacttggtctgacagttaccaatgcttaatcagtgaggcacctatctcagcgatctgtctatttcgttcatccatagttgcctgactccccgtcgtgtagataactacgatacgggagggcttaccatctggccccagtgctgcaatgataccgcgagacccacgctcaccggctccagatttatcagcaataaaccagccagccggaagggccgagcgcagaagtggtcctgcaactttatccgcctccatccagtctattaattgttgccgggaagctagagtaagtagttcgccagttaatagtttgcgcaacgttgttgccattgctacaggcatcgtggtgtcacgctcgtcgtttggtatggcttcattcagctccggttcccaacgatcaaggcgagttacatgatcccccatgttgtgcaaaaaagcggttagctccttcggtcctccgatcgttgtcagaagtaagttggccgcagtgttatcactcatggttatggcagcactgcataattctcttactgtcatgccatccgtaagatgcttttctgtgactggtgagtactcaaccaagtcattctgagaatagtgtatgcggcgaccgagttgctcttgcccggcgtcaatacgggataataccgcgccacatagcagaactttaaaagtgctcatcattggaaaacgttcttcggggcgaaaactctcaaggatcttaccgctgttgagatccagttcgatgtaacccactcgtgcacccaactgatcttcagcatcttttactttcaccagcgtttctgggtgagcaaaaacaggaaggcaaaatgccgcaaaaaagggaataagggcgacacggaaatgttgaatactcatactcttcctttttcaatattattgaagcatttatcagggttattgtctcatgagcggatacatatttgaatgtatttagaaaaataaacaaataggggttccgcgcacatttccccgaaaagtgccacctgacgt

SEQ ID NO: 6 - DNA, 7751 bp, synthetic construct
  source 1..7751: mol_type = other DNA
aagcttggccattgcatacgttgtatccatatcataatatgtacatttatattggctcatgtccaacattaccgccatgttgacattgattattgactagttattaatagtaatcaattacggggtcattagttcatagcccatatatggagttccgcgttacataacttacggtaaatggcccgcctggctgaccgcccaacgacccccgcccattgacgtcaataatgacgtatgttcccatagtaacgccaatagggactttccattgacgtcaatgggtggagtatttacggtaaactgcccacttggcagtacatcaagtgtatcatatgccaagtacgccccctattgacgtcaatgacggtaaatggcccgcctggcattatgcccagtacatgaccttatgggactttcctacttggcagtacatctacgtattagtcatcgctattaccatggtgatgcggttttggcagtacatcaatgggcgtggatagcggtttgactcacggggatttccaagtctccaccccattgacgtcaatgggagtttgttttggcaccaaaatcaacgggactttccaaaatgtcgtaacaactccgccccattgacgcaaatgggcggtaggcgtgtacggtgggaggtctatataagcagagctcgtttagtgaaccggggtctctctggttagaccagatctgagcctgggagctctctggctaactagggaacccactgcttaagcctcaataaagcttgccttgagtgcttcaagtagtgtgtgcccgtctgttgtgtgactctggtaactagagatccctcagacccttttagtcagtgtggaaaatctctagcagtggcgcccgaacagggacctgaaagcgaaagggaaaccagagctctctcgacgcaggactcggcttgctgaagcgcgcacggcaagaggcgaggggcggcgactggtgagtacgccaaaaattttgactagcggaggctagaaggagagagatgggtgcgagagcgtcagtattaagcgggggagaattagatcgcgatgggaaaaaattcggttaaggccagggggaaagaaaaaatataaattaaaacatatagtatgggcaagcagggagctagaacgattcgcagttaatcctggcctgttagaaacatcagaaggctgtagacaaatactgggacagctacaaccatcccttcagacaggatcagaagaacttagatcattatataatacagtagcaaccctctattgtgtgcatcaaaggatagagataaaagacaccaaggaagctttagacaagatagaggaagagcaaaacaaaagtaagaccaccgcacagcaagcggccgctgatcttcagacctggaggaggagatatgagggacaattggagaagtgaattatataaatataaagtagtaaaaattgaaccattaggagtagcacccaccaaggcaaagagaagagtggtgcagagagaaaaaagagcagtgggaataggagctttgttccttgggttcttgggagcagcaggaagcactatgggcgcagcctcaatgacgctgacggtacaggccagacaattattgtctggtatagtgcagcagcagaacaatttgctgagggctattgaggcgcaacagcatctgttgcaactcacagtctggggcatcaagcagctccaggcaagaatcctggctgtggaaagatacctaaaggatcaacagctcctggggatttggggttgctctggaaaactcatttgcaccactgctgtgccttggaatgctagttggagtaataaatctctggaacagattggaatcacacgacctggatggagtgggacagagaaattaacaattacacaagcttaatacactccttaattgaagaatcgcaaaaccagcaagaaaagaatgaacaagaattattggaattagataaatgggcaagtttgtggaattggtttaacataacaaattggctgtggtatataaaattattcataatgatagtaggaggcttggtaggtttaagaatagtttttgctgtactttctatagtgaatagagttaggcagggatattcaccattatcgtttcagacccacctcccaaccccgaggggacccgacaggcccgaaggaatagaagaagaaggtggagagagagacagagacagatccattcgattagtgaacggatctcgacggtatcggttaacttttaaaagaaaaggggggattggggggtacagtgcaggggaaagaatagtagacataatagcaacagacatacaaactaaagaattacaaaaacaaattacaaaaattcaaaattttatcgatcacgagactagcctcgacgatggtcgagtaccgggtaggggaggcgcttttcccaaggcagtctggagcatgcgctttagcagccccgctgggcacttggcgctacacaagtggcctctggcctcgcacacattccacatccaccggtaggcgccaaccggctccgttctttggtggccccttcgcgccaccttctactcctcccctagtcaggaagttcccccccgccccgcagctcgcgtcgtgcaggacgtgacaaatggaagtagcacgtctcactagtctcgtgcagatggacagcaccgctgagcaatggaagcgggtaggcctttggggcagcggccaatagcagctttgctccttcgctttctgggctcagaggctgggaaggggtgggtccgggggcgggctcaggggcgggctcaggggcggggcgggcgcccgaaggtcctccggaggcccggcattctgcacgcttcaaaagcgcacgtctgccgcgctgttctcctcttcctcatctccgggcctttcgacctctagcgggatccaccggtcgccaccatggtgagcaagggcgaggagctgttcaccggggtggtgcccatcctggtcgagctggacggcgacgtaaacggccacaagttcagcgtgtccggcgagggcgagggcgatgccacctacggcaagctgaccctgaagttcatctgcaccaccggcaagctgcccgtgccctggcccaccctcgtgaccaccctgacctacggcgtgcagtgcttcagccgctaccccgaccacatgaagcagcacgacttcttcaagtccgccatgcccgaaggctacgtccaggagcgcaccatcttcttcaaggacgacggcaactacaagacccgcgccgaggtgaagttcgagggcgacaccctggtgaaccgcatcgagctgaagggcatcgacttcaaggaggacggcaacatcctggggcacaagctggagtacaactacaacagccacaacgtctatatcatggccgacaagcagaagaacggcatcaaggtgaacttcaagatccgccacaacatcgaggacggcagcgtgcagctcgccgaccactaccagcagaacacccccatcggcgacggccccgtgctgctgcccgacaaccactacctgagcacccagtccgccctgagcaaagaccccaacgagaagcgcgatcacatggtcctgctggagttcgtgaccgccgccgggatcactctcggcatggacgagctgtacaagtaaagcggcctcgagggaattccgataatcaacctctggattacaaaatttgtgaaagattgactggtattcttaactatgttgctccttttacgctatgtggatacgctgctttaatgcctttgtatcatgctattgcttcccgtatggctttcattttctcctccttgtataaatcctggttgctgtctctttatgaggagttgtggcccgttgtcaggcaacgtggcgtggtgtgcactgtgtttgctgacgcaacccccactggttggggcattgccaccacctgtcagctcctttccgggactttcgctttccccctccctattgccacggcggaactcatcgccgcctgccttgcccgctgctggacaggggctcggctgttgggcactgacaattccgtggtgttgtcggggaagctgacgtcctttccatggctgctcgcctgtgttgccacctggattctgcgcgggacgtccttctgctacgtcccttcggccctcaatccagcggaccttccttcccgcggcctgctgccggctctgcggcctcttccgcgtcttcgccttcgccctcagacgagtcggatctccctttgggccgcctccccgcatcgggaattcgagctcggtacctttaagaccaatgacttacaaggcagctgtagatcttagccactttttaaaagaaaaggggggactggaagggctaattcactcccaacgaagacaagatctgctttttgcttgtactgggtctctctggttagaccagatctgagcctgggagctctctggctaactagggaacccactgcttaagcctcaataaagcttgccttgagtgcttcaagtagtgtgtgcccgtctgttgtgtgactctggtaactagagatccctcagacccttttagtcagtgtggaaaatctctagcagcatctagctagaattaattccgtgtattctatagtgtcacctaaatcgtatgtgtatgatacataaggttatgtattaattgtagccgcgttctaacgacaatatgtacaagcctaattgtgtagcatctggcttactgaagcagaccctatcatctctctcgtaaactgccgtcagagtcggtttggttggacgaaccttctgagtttctggtaacgccgtcccgcacccggaaatggtcagcgaaccaatcagcagggtcatcgctagcctaggcttttgcgtcgagacgtacccaattcgccctatagtgagtcgtattacgcgcgctcactggccgtcgttttacaacgtcgtgactgggaaaaccctggcgttacccaacttaatcgccttgcagcacatccccctttcgccagctggcgtaatagcgaagaggcccgcaccgatcgcccttcccaacagttgcgcagcctgaatggcgaatggcgcgacgcgccctgtagcggcgcattaagcgcggcgggtgtggtggttacgcgcagcgtgaccgctacacttgccagcgccctagcgcccgctcctttcgctttcttcccttcctttctcgccacgttcgccggctttccccgtcaagctctaaatcgggggctccctttagggttccgatttagtgctttacggcacctcgaccccaaaaaacttgattagggtgatggttcacgtagtgggccatcgccctgatagacggtttttcgccctttgacgttggagtccacgttctttaatagtggactcttgttccaaactggaacaacactcaaccctatctcggtctattcttttgatttataagggattttgccgatttcggcctattggttaaaaaatgagctgatttaacaaaaatttaacgcgaattttaacaaaatattaacgtttacaatttcccaggtggcacttttcggggaaatgtgcgcggaacccctatttgtttatttttctaaatacattcaaatatgtatccgctcatgagacaataaccctgataaatgcttcaataatattgaaaaaggaagagtatgagtattcaacatttccgtgtcgcccttattcccttttttgcggcattttgccttcctgtttttgctcacccagaaacgctggtgaaagtaaaagatgctgaagatcagttgggtgcacgagtgggttacatcgaactggatctcaacagcggtaagatccttgagagttttcgccccgaagaacgttttccaatgatgagcacttttaaagttctgctatgtggcgcggtattatcccgtattgacgccgggcaagagcaactcggtcgccgcatacactattctcagaatgacttggttgagtactcaccagtcacagaaaagcatcttacggatggcatgacagtaagagaattatgcagtgctgccataaccatgagtgataacactgcggccaacttacttctgacaacgatcggaggaccgaaggagctaaccgcttttttgcacaacatgggggatcatgtaactcgccttgatcgttgggaaccggagctgaatgaagccataccaaacgacgagcgtgacaccacgatgcctgtagcaatggcaacaacgttgcgcaaactattaactggcgaactacttactctagcttcccggcaacaattaatagactggatggaggcggataaagttgcaggaccacttctgcgctcggcccttccggctggctggtttattgctgataaatctggagccggtgagcgtgggtctcgcggtatcattgcagcactggggccagatggtaagccctcccgtatcgtagttatctacacgacggggagtcaggcaactatggatgaacgaaatagacagatcgctgagataggtgcctcactgattaagcattggtaactgtcagaccaagtttactcatatatactttagattgatttaaaacttcatttttaatttaaaaggatctaggtgaagatcctttttgataatctcatgaccaaaatcccttaacgtgagttttcgttccactgagcgtcagaccccgtagaaaagatcaaaggatcttcttgagatcctttttttctgcgcgtaatctgctgcttgcaaacaaaaaaaccaccgctaccagcggtggtttgtttgccggatcaagagctaccaactctttttccgaaggtaactggcttcagcagagcgcagataccaaatactgtccttctagtgtagccgtagttaggccaccacttcaagaactctgtagcaccgcctacatacctcgctctgctaatcctgttaccagtggctgctgccagtggcgataagtcgtgtcttaccgggttggactcaagacgatagttaccggataaggcgcagcggtcgggctgaacggggggttcgtgcacacagcccagcttggagcgaacgacctacaccgaactgagatacctacagcgtgagctatgagaaagcgccacgcttcccgaagggagaaaggcggacaggtatccggtaagcggcagggtcggaacaggagagcgcacgagggagcttccagggggaaacgcctggtatctttatagtcctgtcgggtttcgccacctctgacttgagcgtcgatttttgtgatgctcgtcaggggggcggagcctatggaaaaacgccagcaacgcggcctttttacggttcctggccttttgctggccttttgctcacatgttctttcctgcgttatcccctgattctgtggataaccgtattaccgcctttgagtgagctgataccgctcgccgcagccgaacgaccgagcgcagcgagtcagtgagcgaggaagcggaagagcgcccaatacgcaaaccgcctctccccgcgcgttggccgattcattaatgcagctggcacgacaggtttcccgactggaaagcgggcagtgagcgcaacgcaattaatgtgagttagctcactcattaggcaccccaggctttacactttatgcttccggctcgtatgttgtgtggaattgtgagcggataacaatttcacacaggaaacagctatgaccatgattacgccaagcgcgcaattaaccctcactaaagggaacaaaagctggagctgc

SEQ ID NO: 7 - protein, 511 aa, synthetic construct
MKCLLYLAFLFIGVNCKFTIVFPHNQKGNWKNVPSNYHYCPSSSDLNWHNDLIGTALQVKMPKSHKAIQADGWMCHASKWVTTCDFRWYGPKYITHSIRSFTPSVEQCKESIEQTKQGTWLNPGFPPQSCGYATVTDAEAVIVQVTPHHVLVDEYTGEWVDSQFINGKCSNYICPTVHNSTTWHSDYKVKGLCDSNLISMDITFFSEDGELSSLGKEGTGFRSNYFAYETGGKACKMQYCKHWGVRLPSGVWFEMADKDLFAAARFPECPEGSSISAPSQTSVDVSLIQDVERILDYSLCQETWSKIRAGLPISPVDLSYLAPKNPGTGPAFTIINGTLKYFETRYIRVDIAAPILSRMVGMISGTTTERELWDDWAPYEDVEIGPNGVLRTSSGYKFPLYMIGHGMLDSDLHLSSKAQVFEHPHIQDAASQLPDDESLFFGDTGLSKNPIELVEGWFSSWKSSIASFFFIIGLIIGLFLVLRVGIHLCIKLKHTKKRQIYTDIEMNRLGK

SEQ ID NO: 8 - protein, 508 aa, synthetic construct
MDWTWILFLVAAATRVHSKFPIYTIPDKLGPWSPIDIHHLSCPNNLVVEDEGCTNLSGFSYMELKVGYISAIKMNGFTCTGVVTEAETYTNFVGYVTTTFKRKHFRPTPDACRAAYNWKMAGDPRYEESLHNPYPDYHWLRTVKTTKESLVIISPSVADLDPYDRSLHSPVFPGGNCSGVAVSSTYCSTNHDYTIWMPENPRLGMSCDIFTNSRGKRASKGSETCGFVDERGLYKSLKGACKLKLCGVLGLRLMDGTWVAMQTSNETKWCPPGQLVNLHDFRSDEIEHLVVEELVKKREECLDALESIMTTKSVSFRRLSHLRKLVPGFGKAYTIFNKTLMEADAHYKSVRTWNEIIPSKGCLRVGGRCHPHVNGVFFNGIILGPDGNVLIPEMQSSLLQQHMELLVSSVIPLMHPLADPSTVFKNGDEAEDFVEVHLPDVHERISGVDLGLPNWGKYVLLSAGALTALMLIIFLMTCWRVGIHLCIKLKHTKKRQIYTDIEMNRLGK

SEQ ID NO: 9 - protein, 1776 aa, synthetic construct
MASNFTQFVLVDNGGTGDVTVAPSNFANGVAEWISSNSRSQAYKVTCSVRQSSAQKRKYTIKVEVPKVATQTVGGVELPVAAWRSYLNMELTIPIFATNSDCELIVKAMQGLLKDGNPIPSAIAANSGIYSQNYPIVQSGLRSRAQASNSAVDGTAGPGSMDSGRDFLTLHGLQDDEDLQALLKGSQLLKVKSSSWRRERFYKLQEDCKTIWQESRKVMRTPESQLFSIEDIQEVRMGHRTEGLEKFARDVPEDRCFSIVFKDQRNTLDLIAPSPADAQHWVLGLHKIIHHSGSMDQRQKLQHWIHSCLRKADKNKDNKMSFKELQNFLKELNIQPRAEFTLAARASVLSGGELDRWEKIRLRPGGKKKYKLKHIVWASRELERFAVNPGLLETSEGCRQILGQLQPSLQTGSEELRSLYNTVATLYCVHQRIEIKDTKEALDKIEEEQNKSKKKAQQAAADTGHSSQVSQNYPIVQNIQGQMVHQAISPRTLNAWVKVVEEKAFSPEVIPMFSALSEGATPQDLNTMLNTVGGHQAAMQMLKETINEEAAEWDRVHPVHAGPIAPGQMREPRGSDIAGTTSTLQEQIGWMTNNPPIPVGEIYKRWIILGLNKIVRMYSPTSILDIRQGPKEPFRDYVDRFYKTLRAEQASQEVKNWMTETLLVQNANPDCKTILKALGPAATLEEMMTACQGVGGPGHKARVLAEAMSQVTNTATIMMQRGNFRNQRKMVKCFNCGKEGHTARNCRAPRKKGCWKCGKEGHQMKDCTERQANFFREDLAFPQGKAREFSSEQTRANSPTRRELQVWGRDNNSLSEAGADRQGTVSFSFPQITLWQRPLVTIKIGGQLKEALLDTGADDTVLEEMNLPGRWKPKMIGGIGGFIKVRQYDQILIEICGHKAIGTVLVGPTPVNIIGRNLLTQIGCTLNFPISPIETVPVKLKPGMDGPKVKQWPLTEEKIKALVEICTEMEKEGKISKIGPENPYNTPVFAIKKKDSTKWRKLVDFRELNKRTQDFWEVQLGIPHPAGLKKKKSVTVLDVGDAYFSVPLDEDFRKYTAFTIPSINNETPGIRYQYNVLPQGWKGSPAIFQSSMTKILEPFKKQNPDIVIYQYMDDLYVGSDLEIGQHRTKIEELRQHLLRWGLTTPDKKHQKEPPFLWMGYELHPDKWTVQPIVLPEKDSWTVNDIQKLVGKLNWASQIYPGIKVRQLCKLLRGTKALTEVIPLTEEAELELAENREILKEPVHGVYYDPSKDLIAEIQKQGQGQWTYQIYQEPFKNLKTGKYARMRGAHTNDVKQLTEAVQKITTESIVIWGKTPKFKLPIQKETWETWWTEYWQATWIPEWEFVNTPPLVKLWYQLEKEPIVGAETFYVDGAANRETKLGKAGYVTNKGRQKVVPLTNTTNQKTELQAIYLALQDSGLEVNIVTDSQYALGIIQAQPDKSESELVNQIIEQLIKKEKVYLAWVPAHKGIGGNEQVDKLVSAGIRKILFLDGIDKAQDEHEKYHSNWRAMASDFNLPPVVAKEIVASCDKCQLKGEAMHGQVDCSPGIWQLVCTHLEGKVILVAVHVASGYIEAEVIPAETGQETAYFLLKLAGRWPVKTIHTDNGSNFTSATVKAACWWAGIKQEFGIPYNPQSQGVVESMNKELKKIIGQVRDQAEHLKTAVQMAVFIHNFKRKGGIGGYSAGERIVDIIATDIQTKELQKQITKIQNFRVYYRDSRNPLWKGPAKLLWKGEGAVVIQDNSDIKVVPRRKAKIIRDYGKQMAGDDCVASRQDED

SEQ ID NO: 10 - RNA, 180 nt, synthetic construct
  source 1..180: mol_type = other RNA
nnnnnnnnnnnnnnnnnnnngtttcagagctaggccaacatgaggatcacccatgtctgcagggcctgctggaaacagcatagcaagttgaaataaggctagtccgttatcaacttggccaacatgaggatcacccatgtctgcagggccgaaaaagtggcaccgagtcggtgctttttt

SEQ ID NO: 11 - RNA, 20 nt, synthetic construct
  source 1..20: mol_type = other RNA
ggccttcatcagcttttcca

SEQ ID NO: 12 - RNA, 20 nt, synthetic construct
  source 1..20: mol_type = other RNA
tgaggaagctgaggaggcgg

SEQ ID NO: 13 - RNA, 20 nt, synthetic construct
  source 1..20: mol_type = other RNA
ggcggcggctgaggaagctg

SEQ ID NO: 14 - RNA, 20 nt, synthetic construct
  source 1..20: mol_type = other RNA
gaaggacttgagggactcga

SEQ ID NO: 15 - RNA, 20 nt, synthetic construct
  source 1..20: mol_type = other RNA
ttcattgccccggtgctgag

SEQ ID NO: 16 - RNA, 20 nt, synthetic construct
  source 1..20: mol_type = other RNA
ggctgaggaagctgaggagg

SEQ ID NO: 17 - RNA, 20 nt, synthetic construct
  source 1..20: mol_type = other RNA
gaccctggaaaagctgatga

SEQ ID NO: 18 - RNA, 20 nt, synthetic construct
  source 1..20: mol_type = other RNA
ggagaccgccatggcgaccc

SEQ ID NO: 19 - RNA, 20 nt, synthetic construct
  source 1..20: mol_type = other RNA
cagcttttccagggtcgcca

SEQ ID NO: 20 - RNA, 20 nt, synthetic construct
  source 1..20: mol_type = other RNA
cttttccagggtcgccatgg

SEQ ID NO: 21 - RNA, 20 nt, synthetic construct
  source 1..20: mol_type = other RNA
aggccttcatcagcttttcc

SEQ ID NO: 22 - RNA, 20 nt, synthetic construct
  source 1..20: mol_type = other RNA
gagtcggcccgaggcctccg

SEQ ID NO: 23 - RNA, 20 nt, synthetic construct
  source 1..20: mol_type = other RNA
ggcggctgaggaagctgagg

SEQ ID NO: 24 - RNA, 20 nt, synthetic construct
  source 1..20: mol_type = other RNA
agcgggcccaaactcacggt

SEQ ID NO: 25 - RNA, 20 nt, synthetic construct
  source 1..20: mol_type = other RNA
agcagcggctgtgcctgcgg

SEQ ID NO: 26 - RNA, 20 nt, synthetic construct
  source 1..20: mol_type = other RNA
ggaagctgaggaggcggcgg

SEQ ID NO: 27 - RNA, 20 nt, synthetic construct
  source 1..20: mol_type = other RNA
gccgggacagggagctgcag

SEQ ID NO: 28 - RNA, 20 nt, synthetic construct
  source 1..20: mol_type = other RNA
tgaggaggcggcggcggcgg

SEQ ID NO: 29 - DNA, 1527 bp, synthetic construct
  source 1..1527: mol_type = other DNA
atggactggacctggatcctgttcctggtggccgccgccacccgcgtgcacagcaagttccctatctacacaattccagataaactgggaccctggagccccattgatattcatcatctgagctgccccaataacctggtggtggaggacgagggctgcaccaatctgagcggcttttcctacatggaactgaaggtgggctacatcagcgccatcaagatgaacggcttcacctgcaccggcgtggtgaccgaggccgagacctacaccaatttcgtgggctacgtgaccaccaccttcaagaggaagcacttccggcccacccccgacgcctgcagagccgcctacaactggaagatggccggcgacccacggtacgaggagagcctgcacaacccttaccccgactatcactggctgaggaccgtgaaaaccaccaaggagagcctcgtgatcatcagccccagcgtggccgacctggacccctacgacagatccctgcacagccccgtgtttcccggcggcaactgtagcggcgtggccgtgagctccacctactgcagcaccaaccacgactacaccatctggatgcccgaaaaccctaggctgggcatgagctgcgacatcttcaccaattccagaggcaagcgggcctccaaggggtccgagacctgtggcttcgtggacgagagaggcctgtacaagagcctgaaaggcgcctgcaagctgaagctgtgcggcgtgctgggcctgaggctgatggacggcacctgggtggcaatgcagaccagcaacgagaccaagtggtgcccccccggccagttggtgaatctgcacgactttaggtctgatgagattgaacacctggtggttgaggaactggtgaaaaagagggaggaatgcctggatgccctggagtccatcatgacaactaaaagcgtgtcttttaggagactgagccacctgagaaagctggtgcctggatttggaaaggcctacactatttttaataagaccctgatggaggctgatgctcactacaagtctgtgagaacttggaatgaaatcatcccttctaaaggctgtctgagagtgggcggcagatgtcacccacacgtgaatggcgtgttctttaacggcattatcctgggcccagatggcaatgtgctgatccctgagatgcagagctccctgctgcagcaacacatggaactgctggtgagcagcgtgatccctctgatgcaccccctggccgatcccagcaccgtgtttaagaatggcgatgaggccgaggattttgtggaggtgcaccttcccgatgtgcacgaacggatctcaggagttgacttgggtctcccgaactgggggaagtatgtattactgagtgcaggggccctgactgccttgatgttgataattttcctgatgacatgctggcgagttggtatccatctttgcattaaattaaagcacaccaagaaaagacagatttatacagacatagagatgaaccgacttggaaagtaa